European Patent Specification EP 3 615 661 B1, published February 11, 2026. Title: Bi- or multi-developed organoid. Applicant: IMBA - INSTITUT FÜR MOLEKULARE BIOTECHNOLOGIE GMBH. The sequence listing filed with the application follows.

SEQUENCE LISTING (22 sequences)

SEQ ID NO: 1 - DNA, 20 bp, Artificial Sequence
  primer
tcccctcttccgatgttgag

SEQ ID NO: 2 - DNA, 19 bp, Artificial Sequence
  primer
gttcttgcagctcggtgac

SEQ ID NO: 3 - DNA, 20 bp, Artificial Sequence
  primer
gaacggcatcaaggtgaact

SEQ ID NO: 4 - DNA, 20 bp, Artificial Sequence
  primer
cttcttggccacgtaacctg

SEQ ID NO: 5 - DNA, 20 bp, Artificial Sequence
  primer
ctacaaggtgaagatgcgcg

SEQ ID NO: 6 - DNA, 20 bp, Artificial Sequence
  primer
tccagcccctcctactctag

SEQ ID NO: 7 - DNA, 20 bp, Artificial Sequence
  primer
tcccctcttccgatgttgag

SEQ ID NO: 8 - DNA, 20 bp, Artificial Sequence
  primer
tccagcccctcctactctag

SEQ ID NO: 9 - DNA, 20 bp, Artificial Sequence
  primer
acgtcccttactccgccaag

SEQ ID NO: 10 - DNA, 21 bp, Artificial Sequence
  primer
agtagatggtgcggggtttcc

SEQ ID NO: 11 - DNA, 20 bp, Artificial Sequence
  primer
tggcccatgtcgcccttcct

SEQ ID NO: 12 - DNA, 20 bp, Artificial Sequence
  primer
gccgacgtggtgccgttgta

SEQ ID NO: 13 - DNA, 19 bp, Artificial Sequence
  primer
caccgccaccacctacaac

SEQ ID NO: 14 - DNA, 20 bp, Artificial Sequence
  primer
caggagttgcgtgctagtga

SEQ ID NO: 15 - DNA, 20 bp, Artificial Sequence
  primer
ccgtctgcaggcaagaacat

SEQ ID NO: 16 - DNA, 19 bp, Artificial Sequence
  primer
gacacacggagcactcgag

SEQ ID NO: 17 - DNA, 19 bp, Artificial Sequence
  primer
gccgtaccaggacaccatg

SEQ ID NO: 18 - DNA, 20 bp, Artificial Sequence
  primer
atgttcttgctcacgtcccc

SEQ ID NO: 19 - DNA, 20 bp, Artificial Sequence
  primer
gggcaccactccactgtatc

SEQ ID NO: 20 - DNA, 21 bp, Artificial Sequence
  primer
cgaagtgcaatggtctttagg

SEQ ID NO: 21 - DNA, 20 bp, Artificial Sequence
  primer
ctcagttcatcgccgtcacc

SEQ ID NO: 22 - DNA, 22 bp, Artificial Sequence
  primer
agccggtgtagatcgtgtcata